European Patent Application EP 4 717 770 A1, published April 1, 2026. Title: 耳蜗毛细胞特异性启动子及其用途. Applicant: 苏州星奥拓维生物技术有限公司. The sequence listing filed with the application follows.

SEQUENCE LISTING (13 sequences)

SEQ ID NO: 1 - DNA, 1351 bp, synthetic construct
  source 1..1351: mol_type = other DNA
acggtactcagctatttgatggcatttttcccaccccatgtgaaattttatttttggaagttatgctagtgacattgcaatatatattgaaatcttcggaggctgccaggttgagcttcaaaactagacttgagaatctttcgtgtatatgcacattcacttgataattgtgtattctatgtagtttaaagtgggatcaagccttttaaaatgtgttattagtacttagaagttgtaaaacagaacttatagaggtttgttactagacactgaaactgcatgacaagtatctggtgtcttaactaattagatagatctgttgtattggttttcttgttggatagaataacagttaatcatttttagaagagttttagattacttgccataaaatttgtatgtctcagctcttgttggtttaggagcagaagtggtgtttagtcccttcccgttaatgttgctgtgctacttcagacagctgaaaacttaatggtattatttcaagttcacataaccctaaaaaaggttttctttgtgtagtaacttgtgcttaaacttttagtcaattaaatgtaggaggttttatttgaaaacataaaatgattctctaaattacatcttgttttaagccaccaaaatgaatgcagtaatttttctttaaaaaaatgatctctgaaaactgtgagacaatgtaaaaagaataagttttaattcccccaaaatcaaaaattgtacttaaaatctcagacaattcactgaacaggtacccaggaacatccaaactgagcagcccacaagacatgcgctcctccctcccgcccacctttatcttaggaaagatttttttttttttaactcgaatccttcaggtgaaaataaagcaacagcagcaacagaaaaaaaaaacgtagtcttcttcagggttaatatcagaagacaagcttgtgcggctttggccaatcagatgcgcccctggcagctataatatagtgctaaaggcagcctctctcacaagctctccaggcttgctaccatttaaaatcagactctttttgtcttttgattgctgtctcgcgacccaactccgatgtgttccgttatcagcggccggcagcctgccattccagcccctgtctgggtggggagcggtggagagtcccccgcagccgcggcgggcaaggttatataggaagagaaagagcgaggcagccagcgagggagagagcgagcgggcgagccggagcgaggaagggaaagcgcaagagagagcgcacacgcacacacccgccgcgcgcactcgcgcacggacccgcacggggacagctcggaagtcatcagttccatgggcgag

SEQ ID NO: 2 - DNA, 762 bp, synthetic construct
  source 1..762: mol_type = other DNA
acggtactcagctatttgatggcatttttcccaccccatgtgaaattttatttttggaagttatgctagtgacattgcaatatatattgaaatcttcggaggctgccaggttgagcttcaaaactagacttgagaatctttcgtgtatatgcacattcacttgataattgtgtattctatgtagtttaaagtgggatcaagccttttaaaatgtgttattagtacttagaagttgtaaaacagaacttatagaggtttgttactagacactgaaactgcatgacaagtatctggtgtcttaactaattagatagatctgttgtattggttttcttgttggatagaataacagttaatcatttttagaagagttttagattacttgccataaaatttgtatgtctcagctcttgttggtttaggagcagaagtggtgtttagtcccttcccgttaatgttgctgtgctacttcagacagctgaaaacttaatggtattatttcaagttcacataaccctaaaaaaggttttctttgtgtagtaacttgtgcttaaacttttagtcaattaaatgtaggaggttttatttgaaaacataaaatgattctctaaattacatcttgttttaagccaccaaaatgaatgcagtaatttttctttaaaaaaatgatctctgaaaactgtgagacaatgtaaaaagaataagttttaattcccccaaaatcaaaaattgtacttaaaatctcagacaattcactgaaca

SEQ ID NO: 3 - DNA, 589 bp, synthetic construct
  source 1..589: mol_type = other DNA
ggtacccaggaacatccaaactgagcagcccacaagacatgcgctcctccctcccgcccacctttatcttaggaaagatttttttttttttaactcgaatccttcaggtgaaaataaagcaacagcagcaacagaaaaaaaaaacgtagtcttcttcagggttaatatcagaagacaagcttgtgcggctttggccaatcagatgcgcccctggcagctataatatagtgctaaaggcagcctctctcacaagctctccaggcttgctaccatttaaaatcagactctttttgtcttttgattgctgtctcgcgacccaactccgatgtgttccgttatcagcggccggcagcctgccattccagcccctgtctgggtggggagcggtggagagtcccccgcagccgcggcgggcaaggttatataggaagagaaagagcgaggcagccagcgagggagagagcgagcgggcgagccggagcgaggaagggaaagcgcaagagagagcgcacacgcacacacccgccgcgcgcactcgcgcacggacccgcacggggacagctcggaagtcatcagttccatgggcgag

SEQ ID NO: 4 - DNA, 708 bp, synthetic construct
  source 1..708: mol_type = other DNA
atggtgtctaagggcgaggaggataacatggccagcctgcctgctacacacgagctgcacatcttcggaagcatcaacggcgtggactttgatatggtgggccagggaaccggcaacccaaacgacggatacgaggagctgaacctgaagagcacaaagggcgatctgcagttctccccctggattctggtgcctcacatcggatacggctttcaccagtacctgccatacccagacggaatgagcccattccaggctgctatggtggatggcagcggctaccaggtgcacaggaccatgcagtttgaggacggcgcctctctgaccgtgaactacagatacacatacgagggaagccacatcaagggcgaggcccaggtgaagggaaccggcttccctgctgacggaccagtgatgaccaactccctgacagccgctgactggtgccggtctaagaaaacataccctaacgataagaccatcatctctacattcaagtggagctacaccacaggaaacggcaagaggtacagatccaccgcccggaccacatacacatttgctaagccaatggccgctaactacctgaagaaccagcccatgtacgtgttccgcaagaccgagctgaagcactccaagacagagctgaacttcaaggagtggcagaaggcctttaccgacgtgatgggaatggatgagctgtacaag

SEQ ID NO: 5 - protein, 236 aa, synthetic construct
MVSKGEEDNMASLPATHELHIFGSINGVDFDMVGQGTGNPNDGYEELNLKSTKGDLQFSPWILVPHIGYGFHQYLPYPDGMSPFQAAMVDGSGYQVHRTMQFEDGASLTVNYRYTYEGSHIKGEAQVKGTGFPADGPVMTNSLTAADWCRSKKTYPNDKTIISTFKWSYTTGNGKRYRSTARTTYTFAKPMAANYLKNQPMYVFRKTELKHSKTELNFKEWQKAFTDVMGMDELYK

SEQ ID NO: 6 - DNA, 941 bp, synthetic construct
  source 1..941: mol_type = other DNA
ccattgacgtcaataatgacgtatgttcccatagtaacgccaatagggactttccattgacgtcaatgggtggagtatttacggtaaactgcccacttggcagtacatcaagtgtatcatatgccaagtacgccccctattgacgtcaatgacggtaaatggcccgcctggcattatgcccagtacatgaccttatgggactttcctacttggcagtacatctacgtattagtcatcgctattaccatggtcgaggtgagccccacgttctgcttcactctccccatctcccccccctccccacccccaattttgtatttatttattttttaattattttgtgcagcgatgggggcggggggggggggggggcgcgcgccgggcggggcggggcggggcgaggggcggggcggggcgaggcggagaggtgcggcggcagccaatcagagcggcgcgctccgaaagtttccttttatggcgaggcggcggcggcggcggccctataaaaagcgaagcgcgcggcgggcgggagtcgctgcgcgctgccttcgccccgtgccccgctccgccgccgcctcgcgccgcccgccccggctctgactgaccgcgttactcccacaggtgagcgggcgggacggcccttctcctccgggctgtaattagcgcttggtttaatgacggcttgtttcttttctgtggctgcgtgaaagccttgaggggctccgggagggccctttgtgcggggggagcggctcggggctgtccgcggggggacggctgccttcgggggggacggggcagggcggggttcggcttctggcgtgtgaccggcggctctagagcctctgctaaccatgttcatgccttcttctttttcctacagctcctgggcaacgtgctggttattgtgctgtctcatcattttggcaaagaattggatc

SEQ ID NO: 7 - DNA, 4461 bp, synthetic construct
  source 1..4461: mol_type = other DNA
cctgcaggcagctgcgcgctcgctcgctcactgaggccgcccgggcaaagcccgggcgtcgggcgacctttggtcgcccggcctcagtgagcgagcgagcgcgcagagagggagtggccaactccatcactaggggttcctgcggccgcacgcgttctcgattctagagaattcgccaccatgaagcggacagctgatggcagcgagttcgagtcccccaagaagaagaggaaggtggagatggtgtctaagggcgaggaggataacatggccagcctgcctgctacacacgagctgcacatcttcggaagcatcaacggcgtggactttgatatggtgggccagggaaccggcaacccaaacgacggatacgaggagctgaacctgaagagcacaaagggcgatctgcagttctccccctggattctggtgcctcacatcggatacggctttcaccagtacctgccatacccagacggaatgagcccattccaggctgctatggtggatggcagcggctaccaggtgcacaggaccatgcagtttgaggacggcgcctctctgaccgtgaactacagatacacatacgagggaagccacatcaagggcgaggcccaggtgaagggaaccggcttccctgctgacggaccagtgatgaccaactccctgacagccgctgactggtgccggtctaagaaaacataccctaacgataagaccatcatctctacattcaagtggagctacaccacaggaaacggcaagaggtacagatccaccgcccggaccacatacacatttgctaagccaatggccgctaactacctgaagaaccagcccatgtacgtgttccgcaagaccgagctgaagcactccaagacagagctgaacttcaaggagtggcagaaggcctttaccgacgtgatgggaatggatgagctgtacaagtgagatatcaagcttatcgataatcaacctctggattacaaaatttgtgaaagattgactggtattcttaactatgttgctccttttacgctatgtggatacgctgctttaatgcctttgtatcatgctattgcttcccgtatggctttcattttctcctccttgtataaatcctggttgctgtctctttatgaggagttgtggcccgttgtcaggcaacgtggcgtggtgtgcactgtgtttgctgacgcaacccccactggttggggcattgccaccacctgtcagctcctttccgggactttcgctttccccctccctattgccacggcggaactcatcgccgcctgccttgcccgctgctggacaggggctcggctgttgggcactgacaattccgtggtgttgtcggggaaatcatcgtcctttccttggctgctcgcctgtgttgccacctggattctgcgcgggacgtccttctgctacgtcccttcggccctcaatccagcggaccttccttcccgcggcctgctgccggctctgcggcctcttccgcgacttcgccttcgccctcagacgagtcggatctccctttgggccgcctccccgcagatctaacttgtttattgcagcttataatggttacaaataaagcaatagcatcacaaatttcacaaataaagcatttttttcactgcattctagttgtggtttgtccaaactcatcaatgtatcttatcatgtctggctagacacgtgcggaccgagcggccgcaggaacccctagtgatggagttggccactccctctctgcgcgctcgctcgctcactgaggccgggcgaccaaaggtcgcccgacgcccgggctttgcccgggcggcctcagtgagcgagcgagcgcgcagctgcctgcaggggcgcctgatgcggtattttctccttacgcatctgtgcggtatttcacaccgcatacgtcaaagcaaccatagtacgcgccctgtagcggcgcattaagcgcggcgggtgtggtggttacgcgcagcgtgaccgctacacttgccagcgccctagcgcccgctcctttcgctttcttcccttcctttctcgccacgttcgccggctttccccgtcaagctctaaatcgggggctccctttagggttccgatttagtgctttacggcacctcgaccccaaaaaacttgatttgggtgatggttcacgtagtgggccatcgccctgatagacggtttttcgccctttgacgttggagtccacgttctttaatagtggactcttgttccaaactggaacaacactcaaccctatctcgggctattcttttgatttataagggattttgccgatttcggcctattggttaaaaaatgagctgatttaacaaaaatttaacgcgaattttaacaaaatattaacgtttacaattttatggtgcactctcagtacaatctgctctgatgccgcatagttaagccagccccgacacccgccaacacccgctgacgcgccctgacgggcttgtctgctcccggcatccgcttacagacaagctgtgaccgtctccgggagctgcatgtgtcagaggttttcaccgtcatcaccgaaacgcgcgagacgaaagggcctcgtgatacgcctatttttataggttaatgtcatgataataatggtttcttagacgtcaggtggcacttttcggggaaatgtgcgcggaacccctatttgtttatttttctaaatacattcaaatatgtatccgctcatgagacaataaccctgataaatgcttcaataatattgaaaaaggaagagtatgagtattcaacatttccgtgtcgcccttattcccttttttgcggcattttgccttcctgtttttgctcacccagaaacgctggtgaaagtaaaagatgctgaagatcagttgggtgcacgagtgggttacatcgaactggatctcaacagcggtaagatccttgagagttttcgccccgaagaacgttttccaatgatgagcacttttaaagttctgctatgtggcgcggtattatcccgtattgacgccgggcaagagcaactcggtcgccgcatacactattctcagaatgacttggttgagtactcaccagtcacagaaaagcatcttacggatggcatgacagtaagagaattatgcagtgctgccataaccatgagtgataacactgcggccaacttacttctgacaacgatcggaggaccgaaggagctaaccgcttttttgcacaacatgggggatcatgtaactcgccttgatcgttgggaaccggagctgaatgaagccataccaaacgacgagcgtgacaccacgatgcctgtagcaatggcaacaacgttgcgcaaactattaactggcgaactacttactctagcttcccggcaacaattaatagactggatggaggcggataaagttgcaggaccacttctgcgctcggcccttccggctggctggtttattgctgataaatctggagccggtgagcgtgggtctcgcggtatcattgcagcactggggccagatggtaagccctcccgtatcgtagttatctacacgacggggagtcaggcaactatggatgaacgaaatagacagatcgctgagataggtgcctcactgattaagcattggtaactgtcagaccaagtttactcatatatactttagattgatttaaaacttcatttttaatttaaaaggatctaggtgaagatcctttttgataatctcatgaccaaaatcccttaacgtgagttttcgttccactgagcgtcagaccccgtagaaaagatcaaaggatcttcttgagatcctttttttctgcgcgtaatctgctgcttgcaaacaaaaaaaccaccgctaccagcggtggtttgtttgccggatcaagagctaccaactctttttccgaaggtaactggcttcagcagagcgcagataccaaatactgtccttctagtgtagccgtagttaggccaccacttcaagaactctgtagcaccgcctacatacctcgctctgctaatcctgttaccagtggctgctgccagtggcgataagtcgtgtcttaccgggttggactcaagacgatagttaccggataaggcgcagcggtcgggctgaacggggggttcgtgcacacagcccagcttggagcgaacgacctacaccgaactgagatacctacagcgtgagctatgagaaagcgccacgcttcccgaagggagaaaggcggacaggtatccggtaagcggcagggtcggaacaggagagcgcacgagggagcttccagggggaaacgcctggtatctttatagtcctgtcgggtttcgccacctctgacttgagcgtcgatttttgtgatgctcgtcaggggggcggagcctatggaaaaacgccagcaacgcggcctttttacggttcctggccttttgctggccttttgctcacatgt

SEQ ID NO: 8 - DNA, 5820 bp, synthetic construct
  source 1..5820: mol_type = other DNA
cctgcaggcagctgcgcgctcgctcgctcactgaggccgcccgggcaaagcccgggcgtcgggcgacctttggtcgcccggcctcagtgagcgagcgagcgcgcagagagggagtggccaactccatcactaggggttcctgcggccgcacgcgttctcgattctagatttacggtactcagctatttgatggcatttttcccaccccatgtgaaattttatttttggaagttatgctagtgacattgcaatatatattgaaatcttcggaggctgccaggttgagcttcaaaactagacttgagaatctttcgtgtatatgcacattcacttgataattgtgtattctatgtagtttaaagtgggatcaagccttttaaaatgtgttattagtacttagaagttgtaaaacagaacttatagaggtttgttactagacactgaaactgcatgacaagtatctggtgtcttaactaattagatagatctgttgtattggttttcttgttggatagaataacagttaatcatttttagaagagttttagattacttgccataaaatttgtatgtctcagctcttgttggtttaggagcagaagtggtgtttagtcccttcccgttaatgttgctgtgctacttcagacagctgaaaacttaatggtattatttcaagttcacataaccctaaaaaaggttttctttgtgtagtaacttgtgcttaaacttttagtcaattaaatgtaggaggttttatttgaaaacataaaatgattctctaaattacatcttgttttaagccaccaaaatgaatgcagtaatttttctttaaaaaaatgatctctgaaaactgtgagacaatgtaaaaagaataagttttaattcccccaaaatcaaaaattgtacttaaaatctcagacaattcactgaacaggtacccaggaacatccaaactgagcagcccacaagacatgcgctcctccctcccgcccacctttatcttaggaaagatttttttttttttaactcgaatccttcaggtgaaaataaagcaacagcagcaacagaaaaaaaaaacgtagtcttcttcagggttaatatcagaagacaagcttgtgcggctttggccaatcagatgcgcccctggcagctataatatagtgctaaaggcagcctctctcacaagctctccaggcttgctaccatttaaaatcagactctttttgtcttttgattgctgtctcgcgacccaactccgatgtgttccgttatcagcggccggcagcctgccattccagcccctgtctgggtggggagcggtggagagtcccccgcagccgcggcgggcaaggttatataggaagagaaagagcgaggcagccagcgagggagagagcgagcgggcgagccggagcgaggaagggaaagcgcaagagagagcgcacacgcacacacccgccgcgcgcactcgcgcacggacccgcacggggacagctcggaagtcatcagttccatgggcgagctagcgaattcgccaccatgaagcggacagctgatggcagcgagttcgagtcccccaagaagaagaggaaggtggagatggtgtctaagggcgaggaggataacatggccagcctgcctgctacacacgagctgcacatcttcggaagcatcaacggcgtggactttgatatggtgggccagggaaccggcaacccaaacgacggatacgaggagctgaacctgaagagcacaaagggcgatctgcagttctccccctggattctggtgcctcacatcggatacggctttcaccagtacctgccatacccagacggaatgagcccattccaggctgctatggtggatggcagcggctaccaggtgcacaggaccatgcagtttgaggacggcgcctctctgaccgtgaactacagatacacatacgagggaagccacatcaagggcgaggcccaggtgaagggaaccggcttccctgctgacggaccagtgatgaccaactccctgacagccgctgactggtgccggtctaagaaaacataccctaacgataagaccatcatctctacattcaagtggagctacaccacaggaaacggcaagaggtacagatccaccgcccggaccacatacacatttgctaagccaatggccgctaactacctgaagaaccagcccatgtacgtgttccgcaagaccgagctgaagcactccaagacagagctgaacttcaaggagtggcagaaggcctttaccgacgtgatgggaatggatgagctgtacaagtgagatatcaagcttatcgataatcaacctctggattacaaaatttgtgaaagattgactggtattcttaactatgttgctccttttacgctatgtggatacgctgctttaatgcctttgtatcatgctattgcttcccgtatggctttcattttctcctccttgtataaatcctggttgctgtctctttatgaggagttgtggcccgttgtcaggcaacgtggcgtggtgtgcactgtgtttgctgacgcaacccccactggttggggcattgccaccacctgtcagctcctttccgggactttcgctttccccctccctattgccacggcggaactcatcgccgcctgccttgcccgctgctggacaggggctcggctgttgggcactgacaattccgtggtgttgtcggggaaatcatcgtcctttccttggctgctcgcctgtgttgccacctggattctgcgcgggacgtccttctgctacgtcccttcggccctcaatccagcggaccttccttcccgcggcctgctgccggctctgcggcctcttccgcgacttcgccttcgccctcagacgagtcggatctccctttgggccgcctccccgcagatctaacttgtttattgcagcttataatggttacaaataaagcaatagcatcacaaatttcacaaataaagcatttttttcactgcattctagttgtggtttgtccaaactcatcaatgtatcttatcatgtctggctagacacgtgcggaccgagcggccgcaggaacccctagtgatggagttggccactccctctctgcgcgctcgctcgctcactgaggccgggcgaccaaaggtcgcccgacgcccgggctttgcccgggcggcctcagtgagcgagcgagcgcgcagctgcctgcaggggcgcctgatgcggtattttctccttacgcatctgtgcggtatttcacaccgcatacgtcaaagcaaccatagtacgcgccctgtagcggcgcattaagcgcggcgggtgtggtggttacgcgcagcgtgaccgctacacttgccagcgccctagcgcccgctcctttcgctttcttcccttcctttctcgccacgttcgccggctttccccgtcaagctctaaatcgggggctccctttagggttccgatttagtgctttacggcacctcgaccccaaaaaacttgatttgggtgatggttcacgtagtgggccatcgccctgatagacggtttttcgccctttgacgttggagtccacgttctttaatagtggactcttgttccaaactggaacaacactcaaccctatctcgggctattcttttgatttataagggattttgccgatttcggcctattggttaaaaaatgagctgatttaacaaaaatttaacgcgaattttaacaaaatattaacgtttacaattttatggtgcactctcagtacaatctgctctgatgccgcatagttaagccagccccgacacccgccaacacccgctgacgcgccctgacgggcttgtctgctcccggcatccgcttacagacaagctgtgaccgtctccgggagctgcatgtgtcagaggttttcaccgtcatcaccgaaacgcgcgagacgaaagggcctcgtgatacgcctatttttataggttaatgtcatgataataatggtttcttagacgtcaggtggcacttttcggggaaatgtgcgcggaacccctatttgtttatttttctaaatacattcaaatatgtatccgctcatgagacaataaccctgataaatgcttcaataatattgaaaaaggaagagtatgagtattcaacatttccgtgtcgcccttattcccttttttgcggcattttgccttcctgtttttgctcacccagaaacgctggtgaaagtaaaagatgctgaagatcagttgggtgcacgagtgggttacatcgaactggatctcaacagcggtaagatccttgagagttttcgccccgaagaacgttttccaatgatgagcacttttaaagttctgctatgtggcgcggtattatcccgtattgacgccgggcaagagcaactcggtcgccgcatacactattctcagaatgacttggttgagtactcaccagtcacagaaaagcatcttacggatggcatgacagtaagagaattatgcagtgctgccataaccatgagtgataacactgcggccaacttacttctgacaacgatcggaggaccgaaggagctaaccgcttttttgcacaacatgggggatcatgtaactcgccttgatcgttgggaaccggagctgaatgaagccataccaaacgacgagcgtgacaccacgatgcctgtagcaatggcaacaacgttgcgcaaactattaactggcgaactacttactctagcttcccggcaacaattaatagactggatggaggcggataaagttgcaggaccacttctgcgctcggcccttccggctggctggtttattgctgataaatctggagccggtgagcgtgggtctcgcggtatcattgcagcactggggccagatggtaagccctcccgtatcgtagttatctacacgacggggagtcaggcaactatggatgaacgaaatagacagatcgctgagataggtgcctcactgattaagcattggtaactgtcagaccaagtttactcatatatactttagattgatttaaaacttcatttttaatttaaaaggatctaggtgaagatcctttttgataatctcatgaccaaaatcccttaacgtgagttttcgttccactgagcgtcagaccccgtagaaaagatcaaaggatcttcttgagatcctttttttctgcgcgtaatctgctgcttgcaaacaaaaaaaccaccgctaccagcggtggtttgtttgccggatcaagagctaccaactctttttccgaaggtaactggcttcagcagagcgcagataccaaatactgtccttctagtgtagccgtagttaggccaccacttcaagaactctgtagcaccgcctacatacctcgctctgctaatcctgttaccagtggctgctgccagtggcgataagtcgtgtcttaccgggttggactcaagacgatagttaccggataaggcgcagcggtcgggctgaacggggggttcgtgcacacagcccagcttggagcgaacgacctacaccgaactgagatacctacagcgtgagctatgagaaagcgccacgcttcccgaagggagaaaggcggacaggtatccggtaagcggcagggtcggaacaggagagcgcacgagggagcttccagggggaaacgcctggtatctttatagtcctgtcgggtttcgccacctctgacttgagcgtcgatttttgtgatgctcgtcaggggggcggagcctatggaaaaacgccagcaacgcggcctttttacggttcctggccttttgctggccttttgctcacatgt

SEQ ID NO: 9 - DNA, 5055 bp, synthetic construct
  source 1..5055: mol_type = other DNA
cctgcaggcagctgcgcgctcgctcgctcactgaggccgcccgggcaaagcccgggcgtcgggcgacctttggtcgcccggcctcagtgagcgagcgagcgcgcagagagggagtggccaactccatcactaggggttcctgcggccgcacgcgttctcgattctagaggtacccaggaacatccaaactgagcagcccacaagacatgcgctcctccctcccgcccacctttatcttaggaaagatttttttttttttaactcgaatccttcaggtgaaaataaagcaacagcagcaacagaaaaaaaaaacgtagtcttcttcagggttaatatcagaagacaagcttgtgcggctttggccaatcagatgcgcccctggcagctataatatagtgctaaaggcagcctctctcacaagctctccaggcttgctaccatttaaaatcagactctttttgtcttttgattgctgtctcgcgacccaactccgatgtgttccgttatcagcggccggcagcctgccattccagcccctgtctgggtggggagcggtggagagtcccccgcagccgcggcgggcaaggttatataggaagagaaagagcgaggcagccagcgagggagagagcgagcgggcgagccggagcgaggaagggaaagcgcaagagagagcgcacacgcacacacccgccgcgcgcactcgcgcacggacccgcacggggacagctcggaagtcatcagttccatgggcgagctagcgaattcgccaccatgaagcggacagctgatggcagcgagttcgagtcccccaagaagaagaggaaggtggagatggtgtctaagggcgaggaggataacatggccagcctgcctgctacacacgagctgcacatcttcggaagcatcaacggcgtggactttgatatggtgggccagggaaccggcaacccaaacgacggatacgaggagctgaacctgaagagcacaaagggcgatctgcagttctccccctggattctggtgcctcacatcggatacggctttcaccagtacctgccatacccagacggaatgagcccattccaggctgctatggtggatggcagcggctaccaggtgcacaggaccatgcagtttgaggacggcgcctctctgaccgtgaactacagatacacatacgagggaagccacatcaagggcgaggcccaggtgaagggaaccggcttccctgctgacggaccagtgatgaccaactccctgacagccgctgactggtgccggtctaagaaaacataccctaacgataagaccatcatctctacattcaagtggagctacaccacaggaaacggcaagaggtacagatccaccgcccggaccacatacacatttgctaagccaatggccgctaactacctgaagaaccagcccatgtacgtgttccgcaagaccgagctgaagcactccaagacagagctgaacttcaaggagtggcagaaggcctttaccgacgtgatgggaatggatgagctgtacaagtgagatatcaagcttatcgataatcaacctctggattacaaaatttgtgaaagattgactggtattcttaactatgttgctccttttacgctatgtggatacgctgctttaatgcctttgtatcatgctattgcttcccgtatggctttcattttctcctccttgtataaatcctggttgctgtctctttatgaggagttgtggcccgttgtcaggcaacgtggcgtggtgtgcactgtgtttgctgacgcaacccccactggttggggcattgccaccacctgtcagctcctttccgggactttcgctttccccctccctattgccacggcggaactcatcgccgcctgccttgcccgctgctggacaggggctcggctgttgggcactgacaattccgtggtgttgtcggggaaatcatcgtcctttccttggctgctcgcctgtgttgccacctggattctgcgcgggacgtccttctgctacgtcccttcggccctcaatccagcggaccttccttcccgcggcctgctgccggctctgcggcctcttccgcgacttcgccttcgccctcagacgagtcggatctccctttgggccgcctccccgcagatctaacttgtttattgcagcttataatggttacaaataaagcaatagcatcacaaatttcacaaataaagcatttttttcactgcattctagttgtggtttgtccaaactcatcaatgtatcttatcatgtctggctagacacgtgcggaccgagcggccgcaggaacccctagtgatggagttggccactccctctctgcgcgctcgctcgctcactgaggccgggcgaccaaaggtcgcccgacgcccgggctttgcccgggcggcctcagtgagcgagcgagcgcgcagctgcctgcaggggcgcctgatgcggtattttctccttacgcatctgtgcggtatttcacaccgcatacgtcaaagcaaccatagtacgcgccctgtagcggcgcattaagcgcggcgggtgtggtggttacgcgcagcgtgaccgctacacttgccagcgccctagcgcccgctcctttcgctttcttcccttcctttctcgccacgttcgccggctttccccgtcaagctctaaatcgggggctccctttagggttccgatttagtgctttacggcacctcgaccccaaaaaacttgatttgggtgatggttcacgtagtgggccatcgccctgatagacggtttttcgccctttgacgttggagtccacgttctttaatagtggactcttgttccaaactggaacaacactcaaccctatctcgggctattcttttgatttataagggattttgccgatttcggcctattggttaaaaaatgagctgatttaacaaaaatttaacgcgaattttaacaaaatattaacgtttacaattttatggtgcactctcagtacaatctgctctgatgccgcatagttaagccagccccgacacccgccaacacccgctgacgcgccctgacgggcttgtctgctcccggcatccgcttacagacaagctgtgaccgtctccgggagctgcatgtgtcagaggttttcaccgtcatcaccgaaacgcgcgagacgaaagggcctcgtgatacgcctatttttataggttaatgtcatgataataatggtttcttagacgtcaggtggcacttttcggggaaatgtgcgcggaacccctatttgtttatttttctaaatacattcaaatatgtatccgctcatgagacaataaccctgataaatgcttcaataatattgaaaaaggaagagtatgagtattcaacatttccgtgtcgcccttattcccttttttgcggcattttgccttcctgtttttgctcacccagaaacgctggtgaaagtaaaagatgctgaagatcagttgggtgcacgagtgggttacatcgaactggatctcaacagcggtaagatccttgagagttttcgccccgaagaacgttttccaatgatgagcacttttaaagttctgctatgtggcgcggtattatcccgtattgacgccgggcaagagcaactcggtcgccgcatacactattctcagaatgacttggttgagtactcaccagtcacagaaaagcatcttacggatggcatgacagtaagagaattatgcagtgctgccataaccatgagtgataacactgcggccaacttacttctgacaacgatcggaggaccgaaggagctaaccgcttttttgcacaacatgggggatcatgtaactcgccttgatcgttgggaaccggagctgaatgaagccataccaaacgacgagcgtgacaccacgatgcctgtagcaatggcaacaacgttgcgcaaactattaactggcgaactacttactctagcttcccggcaacaattaatagactggatggaggcggataaagttgcaggaccacttctgcgctcggcccttccggctggctggtttattgctgataaatctggagccggtgagcgtgggtctcgcggtatcattgcagcactggggccagatggtaagccctcccgtatcgtagttatctacacgacggggagtcaggcaactatggatgaacgaaatagacagatcgctgagataggtgcctcactgattaagcattggtaactgtcagaccaagtttactcatatatactttagattgatttaaaacttcatttttaatttaaaaggatctaggtgaagatcctttttgataatctcatgaccaaaatcccttaacgtgagttttcgttccactgagcgtcagaccccgtagaaaagatcaaaggatcttcttgagatcctttttttctgcgcgtaatctgctgcttgcaaacaaaaaaaccaccgctaccagcggtggtttgtttgccggatcaagagctaccaactctttttccgaaggtaactggcttcagcagagcgcagataccaaatactgtccttctagtgtagccgtagttaggccaccacttcaagaactctgtagcaccgcctacatacctcgctctgctaatcctgttaccagtggctgctgccagtggcgataagtcgtgtcttaccgggttggactcaagacgatagttaccggataaggcgcagcggtcgggctgaacggggggttcgtgcacacagcccagcttggagcgaacgacctacaccgaactgagatacctacagcgtgagctatgagaaagcgccacgcttcccgaagggagaaaggcggacaggtatccggtaagcggcagggtcggaacaggagagcgcacgagggagcttccagggggaaacgcctggtatctttatagtcctgtcgggtttcgccacctctgacttgagcgtcgatttttgtgatgctcgtcaggggggcggagcctatggaaaaacgccagcaacgcggcctttttacggttcctggccttttgctggccttttgctcacatgt

SEQ ID NO: 10 - DNA, 7360 bp, synthetic construct
  source 1..7360: mol_type = other DNA
gcgcgccgatatcgttaacgccccgcgccggccgctctagaactagtggatcccccggaagatcagaagttcctattccgaagttcctattctctagaaagtataggaacttctgatctgcgcagccgccatgccggggttttacgagattgtgattaaggtccccagcgaccttgacgagcatctgcccggcatttctgacagctttgtgaactgggtggccgagaaggaatgggagttgccgccagattctgacatggatctgaatctgattgagcaggcacccctgaccgtggccgagaagctgcagcgcgactttctgacggaatggcgccgtgtgagtaaggccccggaggcccttttctttgtgcaatttgagaagggagagagctacttccacatgcacgtgctcgtggaaaccaccggggtgaaatccatggttttgggacgtttcctgagtcagattcgcgaaaaactgattcagagaatttaccgcgggatcgagccgactttgccaaactggttcgcggtcacaaagaccagaaatggcgccggaggcgggaacaaggtggtggatgagtgctacatccccaattacttgctccccaaaacccagcctgagctccagtgggcgtggactaatatggaacagtatttaagcgcctgtttgaatctcacggagcgtaaacggttggtggcgcagcatctgacgcacgtgtcgcagacgcaggagcagaacaaagagaatcagaatcccaattctgatgcgccggtgatcagatcaaaaacttcagccaggtacatggagctggtcgggtggctcgtggacaaggggattacctcggagaagcagtggatccaggaggaccaggcctcatacatctccttcaatgcggcctccaactcgcggtcccaaatcaaggctgccttggacaatgcgggaaagattatgagcctgactaaaaccgcccccgactacctggtgggccagcagcccgtggaggacatttccagcaatcggatttataaaattttggaactaaacgggtacgatccccaatatgcggcttccgtctttctgggatgggccacgaaaaagttcggcaagaggaacaccatctggctgtttgggcctgcaactaccgggaagaccaacatcgcggaggccatagcccacactgtgcccttctacgggtgcgtaaactggaccaatgagaactttcccttcaacgactgtgtcgacaagatggtgatctggtgggaggaggggaagatgaccgccaaggtcgtggagtcggccaaagccattctcggaggaagcaaggtgcgcgtggaccagaaatgcaagtcctcggcccagatagacccgactcccgtgatcgtcacctccaacaccaacatgtgcgccgtgattgacgggaactcaacgaccttcgaacaccagcagccgttgcaagaccggatgttcaaatttgaactcacccgccgtctggatcatgactttgggaaggtcaccaagcaggaagtcaaagactttttccggtgggcaaaggatcacgtggttgaggtggagcatgaattctacgtcaaaaagggtggagccaagaaaagacccgcccccagtgacgcagatataagtgagcccaaacgggtgcgcgagtcagttgcgcagccatcgacgtcagacgcggaagcttcgatcaactacgcagacaggtaccaaaacaaatgttctcgtcacgtgggcatgaatctgatgctgtttccctgcagacaatgcgagagaatgaatcagaattcaaatatctgcttcactcacggacagaaagactgtttagagtgctttcccgtgtcagaatctcaacccgtttctgtcgtcaaaaaggcgtatcagaaactgtgctacattcatcatatcatgggaaaggtgccagacgcttgcactgcctgcgatctggtcaatgtggatttggatgactgcatctttgaacaataaatgatttaaatcaggtatggctgccgatggttatcttccagattggctcgaggacactctctctgaaggaataagacagtggtggaagctcaaacctggcccaccaccaccaaagcccgcagagcggcataaggacgacagcaggggtcttgtgcttcctgggtacaagtacctcggacccttcaacggactcgacaagggagagccggtcaacgaggcagacgccgcggccctcgagcacgacaaagcctacgaccggcagctcgacagcggagacaacccgtacctcaagtacaaccacgccgacgccgagttccaggagcggctcaaagaagatacgtcttttgggggcaacctcgggcgagcagtcttccaggccaaaaagaggcttcttgaacctcttggtctggttgaggaagcggctaagacggctcctggaaagaagaggcctgtagagcactctcctgtggagccagactcctcctcgggaaccggaaaggcgggccagcagcctgcaagaaaaagattgaattttggtcagactggagacgcagactcagtcccagaccctcaaccaatcggagaacctcccgcagccccctcaggtgtgggatctcttacaatggctgcaggcggtggcgcaccaatggcagacaataacgagggcgccgacggagtgggtaattcctcgggaaattggcattgcgattccacatggatgggcgacagagtcatcaccaccagcacccgaacctgggccctgcccacctacaacaaccacctctacaagcaaatctccaacagcacatctggaggatcttcaaatgacaacgcctacttcggctacagcaccccctgggggtattttgactttaacagattccactgccacttttcaccacgtgactggcagcgactcatcaacaacaactggggattccggcccaagagactcagcttcaagctcttcaacatccaggtcaaggaggtcacgcagaatgaaggcaccaagaccatcgccaataacctcaccagcaccatccaggtgtttacggactcggagtaccagctgccgtacgttctcggctctgcccaccagggctgcctgcctccgttcccggcggacgtgttcatgattccccagtacggctacctaacactcaacaacggtagtcaggccgtgggacgctcctccttctactgcctggaatactttccttcgcagatgctgagaaccggcaacaacttccagtttacttacaccttcgaggacgtgcctttccacagcagctacgcccacagccagagcttggaccggctgatgaatcctctgattgaccagtacctgtactacttgtctcggactcaaacaacaggaggcacgacaaatacgcagactctgggcttcagccaaggtgggcctaatacaatggccaatcaggcaaagaactggctgccaggaccctgttaccgccagcagcgagtatcaaagacatctgcggataacaacaacagtgaatactcgtggactggagctaccaagtaccacctcaatggcagagactctctggtgaatccgggcccggccatggcaagccacaaggacgatgaagaaaagttttttcctcagagcggggttctcatctttgggaagcaaggctcagagaaaacaaatgtggacattgaaaaggtcatgattacagacgaagaggaaatcaggacaaccaatcccgtggctacggagcagtatggttctgtatctaccaacctccagagaggcaacgatgggactttggcggtgccttttaagagacaagcagctaccgcagatgtcaacacacaaggcgttcttccaggcatggtctggcaggacagagatgtgtaccttcaggggcccatctgggcaaagattccacacacggacggacattttcacccctctcccctcatgggtggattcggacttaaacaccctccgcctcagatcctgatcaagaacacgcctgtacctgcggatcctccgaccaccttcaaccagtcaaagctgaactctttcatcacccagtattctactggccaagtcagcgtggagatcgagtgggagctgcagaaggaaaacagcaagcgctggaaccccgagatccagtacacctccaactactacaaatctacaagtgtggactttgctgttaatacagaaggcgtgtactctgaaccccgccccattggcacccgttacctcacccgtaatctgtaattgcttgttaatcaataaaccgtttaattcgtttcagttgaactttggtctctgcgtatttctttcttatctagtttccatggctacgtagataagtagcatggcgggttaatcattaactacagcccgggcgtttaaacagcgggcggaggggtggagtcgtgacgtgaattacgtcatagggttagggaggtcctgtattagaggtcacgtgagtgttttgcgacattttgcgacaccatgtggtctcgctgggggggggggcccgagtgagcacgcagggtctccattttgaagcgggaggtttgaacgagcgctggcgcgctcactggccgtcgttttacaacgtcgtgactgggaaaaccctggcgttacccaacttaatcgccttgcagcacatccccctttcgccagctggcgtaatagcgaagaggcccgcaccgatcgcccttcccaacagttgcgcagcctgaatggcgaatggaaattgtaagcgttaatattttgttaaaattcgcgttaaatttttgttaaatcagctcatttttttaaccaataggccgaaatcggcaaaatcccttataaatcaaaagaatagaccgagatagggttgagtgttgttccagtttggaacaagagtccactattaagaacgtggactccaacgtcaaagggcgaaaaaccgtctatcagggcgatggcccactacgtgaaccatcaccctaatcaagttttttggggtcgaggtgccgtaaagcactaaatcggaaccctaaagggagcccccgatttagagcttgacggggaaagccggcgaacgtggcgagaaaggaagggaagaaagcgaaaggagcgggcgctagggcgctggcaagtgtagcggtcacgctgcgcgtaaccaccacacccgccgcgcttaatgcgccgctacagggcgcgtcaggtggcacttttcggggaaatgtgcgcggaacccctatttgtttatttttctaaatacattcaaatatgtatccgctcatgagacaataaccctgataaatgcttcaataatattgaaaaaggaagagtatgagtattcaacatttccgtgtcgcccttattcccttttttgcggcattttgccttcctgtttttgctcacccagaaacgctggtgaaagtaaaagatgctgaagatcagttgggtgcacgagtgggttacatcgaactggatctcaacagcggtaagatccttgagagttttcgccccgaagaacgttttccaatgatgagcacttttaaagttctgctatgtggcgcggtattatcccgtattgacgccgggcaagagcaactcggtcgccgcatacactattctcagaatgacttggttgagtactcaccagtcacagaaaagcatcttacggatggcatgacagtaagagaattatgcagtgctgccataaccatgagtgataacactgcggccaacttacttctgacaacgatcggaggaccgaaggagctaaccgcttttttgcacaacatgggggatcatgtaactcgccttgatcgttgggaaccggagctgaatgaagccataccaaacgacgagcgtgacaccacgatgcctgtagcaatggcaacaacgttgcgcaaactattaactggcgaactacttactctagcttcccggcaacaattaatagactggatggaggcggataaagttgcaggaccacttctgcgctcggcccttccggctggctggtttattgctgataaatctggagccggtgagcgtgggtctcgcggtatcattgcagcactggggccagatggtaagccctcccgtatcgtagttatctacacgacggggagtcaggcaactatggatgaacgaaatagacagatcgctgagataggtgcctcactgattaagcattggtaactgtcagaccaagtttactcatatatactttagattgatttaaaacttcatttttaatttaaaaggatctaggtgaagatcctttttgataatctcatgaccaaaatcccttaacgtgagttttcgttccactgagcgtcagaccccgtagaaaagatcaaaggatcttcttgagatcctttttttctgcgcgtaatctgctgcttgcaaacaaaaaaaccaccgctaccagcggtggtttgtttgccggatcaagagctaccaactctttttccgaaggtaactggcttcagcagagcgcagataccaaatactgttcttctagtgtagccgtagttaggccaccacttcaagaactctgtagcaccgcctacatacctcgctctgctaatcctgttaccagtggctgctgccagtggcgataagtcgtgtcttaccgggttggactcaagacgatagttaccggataaggcgcagcggtcgggctgaacggggggttcgtgcacacagcccagcttggagcgaacgacctacaccgaactgagatacctacagcgtgagctatgagaaagcgccacgcttcccgaagggagaaaggcggacaggtatccggtaagcggcagggtcggaacaggagagcgcacgagggagcttccagggggaaacgcctggtatctttatagtcctgtcgggtttcgccacctctgacttgagcgtcgatttttgtgatgctcgtcaggggggcggagcctatggaaaaacgccagcaacgcggcctttttacggttcctggccttttgctggccttttgctcacatgttctttcctgcgttatcccctgattctgtggataaccgtattaccgcctttgagtgagctgataccgctcgccgcagccgaacgaccgagcgcagcgagtcagtgagcgaggaagcggaagagcgcccaatacgcaaaccgcctctccccgcgcgttggccgattcattaatgcagctggcacgacaggtttcccgactggaaagcgggcagtgagcgcaacgcaattaatgtgagttagctcactcattaggcaccccaggctttacactttatgcttccggctcgtatgttgtgtggaattgtgagcggataacaatttcacacaggaaacagctatgaccatgattacgccaa

SEQ ID NO: 11 - DNA, 5000 bp, synthetic construct
  source 1..5000: mol_type = other DNA
cctgcaggcagctgcgcgctcgctcgctcactgaggccgcccgggcaaagcccgggcgtcgggcgacctttggtcgcccggcctcagtgagcgagcgagcgcgcagagagggagtggccaactccatcactaggggttcctgcggccgcacgcgttctcgagcgcgttgacattgattattgactagttattaatagtaatcaattacggggtcattagttcatagcccatatatggagttccgcgttacataacttacggtaaatggcccgcctggctgaccgcccaacgacccccgcccattgacgtcaataatgacgtatgttcccatagtaacgccaatagggactttccattgacgtcaatgggtggagtatttacggtaaactgcccacttggcagtacatcaagtgtatcatatgccaagtacgccccctattgacgtcaatgacggtaaatggcccgcctggcattatgcccagtacatgaccttatgggactttcctacttggcagtacatctacgtattagtcatcgctattaccatggtgatgcggttttggcagtacatcaatgggcgtggatagcggtttgactcacggggatttccaagtctccaccccattgacgtcaatgggagtttgttttggcaccaaaatcaacgggactttccaaaatgtcgtaacaactccgccccattgacgcaaatgggcggtaggcgtgtacggtgggaggtctatataagcagagctggtttagtgaaccgtcagatccgctagagatccgaattgctagcgccaccatggccttgctcatccacctcaagacagtctcggagctgcggggcaggggcgaccggatcgccaaagtgactttccgagggcaatccttctactctcgggtcctggagaactgtgaggatgtggctgactttgatgagacatttcggtggccggtggccagcagcatcgacagaaatgagatgctggagattcaggttttcaactacagcaaagtcttcagcaacaagctcatcgggaccttccgcatggtgctgcagaaggtggtagaggagagccatgtggaggtgactgacacgctgattgatgacaacaatgctatcatcaagaccagcctgtgcgtggaggtccggtatcaggccactgacggcacagtgggctcctgggacgatggggacttcctgggagatgagtctcttcaagaggaagagaaggacagccaagagacggatggactgctcccaggctcccggcccagctcccggcccccaggagagaagagcttccggagagccgggaggagcgtgttctccgccatgaagctcggcaaaaaccggtctcacaaggaggagccccaaagaccagatgaaccggcggtgctggagatggaagaccttgaccatctggccattcggctaggagatggactggatcccgactcggtgtctctagcctcagtcacagctctcaccactaatgtctccaacaagcgatctaagccagacattaagatggagccaagtgctgggcggcccatggattaccaggtcagcatcacggtgatcgaggcccggcagctggtgggcttgaacatggaccctgtggtgtgcgtggaggtgggtgacgacaagaagtacacatccatgaaggagtccactaactgcccctattacaacgagtacttcgtcttcgacttccatgtctctccggatgtcatgtttgacaagatcatcaagatttcggtgattcactccaagaacctgctgcgcagtggcaccctggtgggctccttcaaaatggacgtgggaaccgtgtactcgcagccagagcaccagttccatcacaagtgggccatcctgtctgaccccgatgacatctcctcggggctgaagggctacgtgaagtgtgacgttgccgtggtgggcaaaggggacaacatcaagacgccccacaaggccaatgagaccgacgaagatgacattgaggggaacttgctgctccccgagggggtgccccccgaacgccagtgggcccggttctatgtgaaaatttaccgagcagaggggctgccccgtatgaacacaagcctcatggccaatgtaaagaaggctttcatcggtgaaaacaaggacctcgtggacccctacgtgcaagtcttctttgctggccagaagggcaagacttcagtgcagaagagcagctatgagcccctgtggaatgagcaggtcgtctttacagacctcttccccccactctgcaaacgcatgaaggtgcagatccgagactcggacaaggtcaacgacgtggccatcggcacccacttcattgacctgcgcaagatttctaatgacggagacaaaggcttcctgcccacactgggcccagcctgggtgaacatgtacggctccacacgtaactacacgctgctggatgagcatcaggacctgaacgagggcctgggggagggtgtgtccttccgggcccggctcctgctgggcctggctgtggagatcgtagacacctccaaccctgagctcaccagctccacagaggtgcaggtggagcaggccacgcccatctcggagagctgtgcaggtaaaatggaagaattctttctctttggagccttcctggaggcctcaatgatcgaccggagaaacggagacaagcccatcacctttgaggtcaccataggcaactatgggaacgaagttgatggcctgtcccggccccagcggcctcggccccggaaggagccgggggatgaggaagaagtagacctgattcagaacgcaagtgatgacgaggccggtgatgccggggacctggcctcagtctcctccactccaccaatgcggccccaggtcaccgacaggaactacttccatctgccctacctggagcgaaagccctgcatctacatcaagagctggtggccggaccagcgccgccgcctctacaatgccaacatcatggaccacattgccgacaagctggtaagtatcaaggttacaagacaggtttaaggagaccaatagaaactgggcttgtcgagacagagaagactcttgcgtttctgggattttgccgatttcggcctattggttaaaaaatgagctgatttaacaaaaatttaacgcgaattttaacaaaatcacgtgcggaccgagcggccgcaggaacccctagtgatggagttggccactccctctctgcgcgctcgctcgctcactgaggccgggcgaccaaaggtcgcccgacgcccgggctttgcccgggcggcctcagtgagcgagcgagcgcgcagctgcctgcaggggcgcctgatgcggtattttctccttacgcatctgtgcggtatttcacaccgcatacgtcaaagcaaccatagtacgcgccctgtagcggcgcattaagcgcggcgggtgtggtggttacgcgcagcgtgaccgctacacttgccagcgccctagcgcccgctcctttcgctttcttcccttcctttctcgccacgttcgccggctttccccgtcaagctctaaatcgggggctccctttagggttccgatttagtgctttacggcacctcgaccccaaaaaacttgatttgggtgatggttcacgtagtgggccatcgccctgatagacggtttttcgccctttgacgttggagtccacgttctttaatagtggactcttgttccaaactggaacaacactcaaccctatctcgggctattcttttgatttataagggattttgccgatttcggcctattggttaaaaaatgagctgatttaacaaaaatttaacgcgaattttaacaaaatattaacgtttacaattttatggtgcactctcagtacaatctgctctgatgccgcatagttaagccagccccgacacccgccaacacccgctgacgcgccctgacgggcttgtctgctcccggcatccgcttacagacaagctgtgaccgtctccgggagctgcatgtgtcagaggttttcaccgtcatcaccgaaacgcgcgagacgaaagggcctcgtgatacgcctatttttataggttaatgtcatgataataatggtttcttagacgtcaggtggcacttttcggggaaatgtgcgcggaacccctatttgtttatttttctaaatacattcaaatatgtatccgctcatgagacaataaccctgataaatgcttcaataatattgaaaaaggaagagtatgagtattcaacatttccgtgtcgcccttattcccttttttgcggcattttgccttcctgtttttgctcacccagaaacgctggtgaaagtaaaagatgctgaagatcagttgggtgcacgagtgggttacatcgaactggatctcaacagcggtaagatccttgagagttttcgccccgaagaacgttttccaatgatgagcacttttaaagttctgctatgtggcgcggtattatcccgtattgacgccgggcaagagcaactcggtcgccgcatacactattctcagaatgacttggttgagtactcaccagtcacagaaaagcatcttacggatggcatgacagtaagagaattatgcagtgctgccataaccatgagtgataacactgcggccaacttacttctgacaacgatcggaggaccgaaggagctaaccgcttttttgcacaacatgggggatcatgtaactcgccttgatcgttgggaaccggagctgaatgaagccataccaaacgacgagcgtgacaccacgatgcctgtagcaatggcaacaacgttgcgcaaactattaactggcgaactacttactctagcttcccggcaacaattaatagactggatggaggcggataaagttgcaggaccacttctgcgctcggcccttccggctggctggtttattgctgataaatctggagccggtgagcgtgggtctcgcggtatcattgcagcactggggcc

SEQ ID NO: 12 - DNA, 5000 bp, synthetic construct
  source 1..5000: mol_type = other DNA
cctgcaggcagctgcgcgctcgctcgctcactgaggccgcccgggcaaagcccgggcgtcgggcgacctttggtcgcccggcctcagtgagcgagcgagcgcgcagagagggagtggccaactccatcactaggggttcctgcggccgcacgcgtgggattttgccgatttcggcctattggttaaaaaatgagctgatttaacaaaaatttaacgcgaattttaacaaaatgataggcacctattggtcttactgacatccactttgcctttctctccacaggaagaaggcctgaacgacatacaggagatgatcaaaacggagaagtcctaccctgagcgtcgcctgcggggcgtcctggaggagctgagctgtggctgctgccgcttcctctccctcgctgacaaggaccagggccactcatcccgcaccaggcttgaccgggagcgcctcaagtcctgcatgagggagctggaaaacatggggcagcaggccaggatgctgcgggcccaggtgaagcggcacacggtgcgggacaagctgaggctgtgccagaacttcctgcagaagctgcgcttcctggcggacgagccccagcacagcattcccgacatcttcatctggatgatgagcaacaacaagcgtgtcgcctatgcccgtgtgccctccaaggacctgctcttctccatcgtggaggaggagactggcaaggactgcgccaaggtcaagacgctcttccttaagctgccagggaagcggggcttcggctcggcaggctggacagtgcaggccaaggtggagctgtacctgtggctgggcctcagcaaacagcgcaaggagttcctgtgcggcctgccctgtggcttccaggaggtcaaggcagcccagggcctgggcctgcatgccttcccacccgtcagcctggtctacaccaagaagcaggcgttccagctccgagcgcacatgtaccaggcccgcagcctctttgccgccgacagcagcggactctcagacccctttgcccgcgtcttcttcatcaatcagagtcagtgcacagaggtgctgaatgagaccctgtgtcccacctgggaccagatgctggtgttcgacaacctggagctctatggtgaagctcatgagctgagggacgatccgcccatcattgtcattgaaatctatgaccaggattccatgggcaaagctgacttcatgggccggaccttcgccaaacccctggtgaagatggcagacgaggcgtactgcccaccccgcttcccacctcagctcgagtactaccagatctaccgtggcaacgccacagctggagacctgctggcggccttcgagctgctgcagattggaccagcagggaaggctgacctgccccccatcaatggcccggtggacgtggaccgaggtcccatcatgcccgtgcccatgggcatccggcccgtgctcagcaagtaccgagtggaggtgctgttctggggcctacgggacctaaagcgggtgaacctggcccaggtggaccggccacgggtggacatcgagtgtgcagggaagggggtgcagtcgtccctgatccacaattataagaagaaccccaacttcaacaccctcgtcaagtggtttgaagtggacctcccagagaacgagctgctgcacccgcccttgaacatccgtgtggtggactgccgggccttcggtcgctacacactggtgggctcccatgccgtcagctccctgcgacgcttcatctaccggcccccagaccgctcggcccccagctggaacaccacggtcaggcttctccggcgctgccgtgtgctgtgcaatgggggctcctcctctcactccacaggggaggttgtggtgactatggagccagaggtacccatcaagaaactggagaccatggtgaagctggacgcgacttctgaagctgttgtcaaggtggatgtggctgaggaggagaaggagaagaagaagaagaagaagggcactgcggaggagccagaggaggaggagccagacgagagcatgctggactggtggtccaagtactttgcctccattgacaccatgaaggagcaacttcgacaacaagagccctctggaattgacttggaggagaaggaggaagtggacaataccgagggcctgaaggggtcaatgaagggcaaggagaaggcaagggctgccaaagaggagaagaagaagaaaactcagagctctggctctggccaggggtccgaggcccccgagaagaagaaacccaagattgatgagcttaaggtataccccaaagagctggagtccgagtttgataactttgaggactggctgcacactttcaacttgcttcggggcaagaccggggatgatgaggatggctccaccgaggaggagcgcattgtgggacgcttcaagggctccctctgcgtgtacaaagtgccactcccagaggacgtgtcccgggaagccggctacgactccacctacggcatgttccagggcatcccgagcaatgaccccatcaatgtgctggtccgagtctatgtggtccgggccacggacctgcaccctgctgacatcaacggcaaagctgacccctacatcgccatccggctaggcaagactgacatccgcgacaaggagaactacatctccaagcagctcaaccctgtctttgggaagtcctttgacatcgaggcctccttccccatggaatccatgctgacggtggctgtgtatgactgggacctggtgggcactgatgacctcattggggaaaccaagatcgacctggagaaccgcttctacagcaagcaccgcgccacctgcggcatcgcccagacctactccacacatggctacaatatctggcgggaccccatgaagcccagccagatcctgacccgcctctgcaaagacggcaaagtggacggcccccactttgggccccctgggagagtgaaggtggccaaccgcgtcttcactgggccctctgagattgaggacgagaacggtcagaggaagcccacagacgagcatgtggcgctgttggccctgaggcactgggaggacatcccccgcgcaggctgccgcctggtgccagagcatgtggagacgaggccgctgctcaaccccgacaagccgggcatcgagcagggccgcctggagctgtgggtggacatgttccccatggacatgccagcccctgggacgcctctggacatctcacctcggaagcccaagaagtacgagctgcgggtcatcatctggaacacagatgaggtggtcttggaggacgacgacttcttcacaggggagaagtccagtgacatcttcgtgagggggtggctgaagggccagcaggaggacaagcaggacacagacgtccactaccactccctcactggcgagggcaacttcaactggcgctacctgttccccttcgactacctggcggcggaggagaagatcgtcatctccaagaaggagtccatgttctcctgggacgagaccgagtacaagatccccgcgcggctcaccctgcagatctgggatgcggaccacttctccgctgacgacttcctgggggccatcgagctggacctgaaccggttcccgcggggcgcaaagacagccaagcagtgcaccatggagatggccaccggggaggtggacgtgcccctcgtgtccatcttcaagcaaaagcgcgtcaaaggctggtggcccctcctggcccgcaatgagaacgatgagtttgagctcacgggcaaggtggaggctgagctgcatttactgacagcagaggaggcagagaagaacccagtgggcctggcccgcaatgaacctgaccccctagagaaacccaaccggcccgacacggccttcgtctggttcctcaaccctctcaagtccatcaagtacctcatctgcacccggtacaagtggctcatcatcaagatcgtgctggcgctgttggggctgctcatgttggggctcttcctctacagcctccctggctacatggtcaaaaagctccttggggcaggatccggttcctatccatatgacgttccagattacgcttgagatatcaagcttatcgataatcaacctctggattacaaaatttgtgaaagattgactggtattcttaactatgttgctccttttacgctatgtggatacgctgctttaatgcctttgtatcatgctattgcttcccgtatggctttcattttctcctccttgtataaatcctggttgctgtctctttatgaggagttgtggcccgttgtcaggcaacgtggcgtggtgtgcactgtgtttgctgacgcaacccccactggttggggcattgccaccacctgtcagctcctttccgggactttcgctttccccctccctattgccacggcggaactcatcgccgcctgccttgcccgctgctggacaggggctcggctgttgggcactgacaattccgtggtgttgtcggggaaatcatcgtcctttccttggctgctcgcctgtgttgccacctggattctgcgcgggacgtccttctgctacgtcccttcggccctcaatccagcggaccttccttcccgcggcctgctgccggctctgcggcctcttccgcgacttcgccttcgccctcagacgagtcggatctccctttgggccgcctccccgcagatctaacttgtttattgcagcttataatggttacaaataaagcaatagcatcacaaatttcacaaataaagcatttttttcactgcattctagttgtggtttgtccaaactcatcaatgtatcttatcatgtctggctagacacgtgcggaccgagcggccgcaggaacccctagtgatggagttggccactccctctctgcgcgctcgctcgctcactgaggccgggcgaccaaaggtcgcccgacgcccgggctttgcccgggcggcctcagtgagcgagcgagcgc

SEQ ID NO: 13 - DNA, 5000 bp, synthetic construct
  source 1..5000: mol_type = other DNA
cctgcaggcagctgcgcgctcgctcgctcactgaggccgcccgggcaaagcccgggcgtcgggcgacctttggtcgcccggcctcagtgagcgagcgagcgcgcagagagggagtggccaactccatcactaggggttcctgcggccgcacgcgttctcgagcgcgttacggtactcagctatttgatggcatttttcccaccccatgtgaaattttatttttggaagttatgctagtgacattgcaatatatattgaaatcttcggaggctgccaggttgagcttcaaaactagacttgagaatctttcgtgtatatgcacattcacttgataattgtgtattctatgtagtttaaagtgggatcaagccttttaaaatgtgttattagtacttagaagttgtaaaacagaacttatagaggtttgttactagacactgaaactgcatgacaagtatctggtgtcttaactaattagatagatctgttgtattggttttcttgttggatagaataacagttaatcatttttagaagagttttagattacttgccataaaatttgtatgtctcagctcttgttggtttaggagcagaagtggtgtttagtcccttcccgttaatgttgctgtgctacttcagacagctgaaaacttaatggtattatttcaagttcacataaccctaaaaaaggttttctttgtgtagtaacttgtgcttaaacttttagtcaattaaatgtaggaggttttatttgaaaacataaaatgattctctaaattacatcttgttttaagccaccaaaatgaatgcagtaatttttctttaaaaaaatgatctctgaaaactgtgagacaatgtaaaaagaataagttttaattcccccaaaatcaaaaattgtacttaaaatctcagacaattcactgaacaggtacccaggaacatccaaactgagcagcccacaagacatgcgctcctccctcccgcccacctttatcttaggaaagatttttttttttttaactcgaatccttcaggtgaaaataaagcaacagcagcaacagaaaaaaaaaacgtagtcttcttcagggttaatatcagaagacaagcttgtgcggctttggccaatcagatgcgcccctggcagctataatatagtgctaaaggcagcctctctcacaagctctccaggcttgctaccatttaaaatcagactctttttgtcttttgattgctgtctcgcgacccaactccgatgtgttccgttatcagcggccggcagcctgccattccagcccctgtctgggtggggagcggtggagagtcccccgcagccgcggcgggcaaggttatataggaagagaaagagcgaggcagccagcgagggagagagcgagcgggcgagccggagcgaggaagggaaagcgcaagagagagcgcacacgcacacacccgccgcgcgcactcgcgcacggacccgcacggggacagctcggaagtcatcagttccatgggcgagggtttagtgaaccgtcagatccgctagagatccgaattgctagcgccaccatggccttgctcatccacctcaagacagtctcggagctgcggggcaggggcgaccggatcgccaaagtgactttccgagggcaatccttctactctcgggtcctggagaactgtgaggatgtggctgactttgatgagacatttcggtggccggtggccagcagcatcgacagaaatgagatgctggagattcaggttttcaactacagcaaagtcttcagcaacaagctcatcgggaccttccgcatggtgctgcagaaggtggtagaggagagccatgtggaggtgactgacacgctgattgatgacaacaatgctatcatcaagaccagcctgtgcgtggaggtccggtatcaggccactgacggcacagtgggctcctgggacgatggggacttcctgggagatgagtctcttcaagaggaagagaaggacagccaagagacggatggactgctcccaggctcccggcccagctcccggcccccaggagagaagagcttccggagagccgggaggagcgtgttctccgccatgaagctcggcaaaaaccggtctcacaaggaggagccccaaagaccagatgaaccggcggtgctggagatggaagaccttgaccatctggccattcggctaggagatggactggatcccgactcggtgtctctagcctcagtcacagctctcaccactaatgtctccaacaagcgatctaagccagacattaagatggagccaagtgctgggcggcccatggattaccaggtcagcatcacggtgatcgaggcccggcagctggtgggcttgaacatggaccctgtggtgtgcgtggaggtgggtgacgacaagaagtacacatccatgaaggagtccactaactgcccctattacaacgagtacttcgtcttcgacttccatgtctctccggatgtcatgtttgacaagatcatcaagatttcggtgattcactccaagaacctgctgcgcagtggcaccctggtgggctccttcaaaatggacgtgggaaccgtgtactcgcagccagagcaccagttccatcacaagtgggccatcctgtctgaccccgatgacatctcctcggggctgaagggctacgtgaagtgtgacgttgccgtggtgggcaaaggggacaacatcaagacgccccacaaggccaatgagaccgacgaagatgacattgaggggaacttgctgctccccgagggggtgccccccgaacgccagtgggcccggttctatgtgaaaatttaccgagcagaggggctgccccgtatgaacacaagcctcatggccaatgtaaagaaggctttcatcggtgaaaacaaggacctcgtggacccctacgtgcaagtcttctttgctggccagaagggcaagacttcagtgcagaagagcagctatgagcccctgtggaatgagcaggtcgtctttacagacctcttccccccactctgcaaacgcatgaaggtgcagatccgagactcggacaaggtcaacgacgtggccatcggcacccacttcattgacctgcgcaagatttctaatgacggagacaaaggcttcctgcccacactgggcccagcctgggtgaacatgtacggctccacacgtaactacacgctgctggatgagcatcaggacctgaacgagggcctgggggagggtgtgtccttccgggcccggctcctgctgggcctggctgtggagatcgtagacacctccaaccctgagctcaccagctccacagaggtgcaggtggagcaggccacgcccatctcggagagctgtgcaggtaaaatggaagaattctttctctttggagccttcctggaggcctcaatgatcgaccggagaaacggagacaagcccatcacctttgaggtcaccataggcaactatgggaacgaagttgatggcctgtcccggccccagcggcctcggccccggaaggagccgggggatgaggaagaagtagacctgattcagaacgcaagtgatgacgaggccggtgatgccggggacctggcctcagtctcctccactccaccaatgcggccccaggtcaccgacaggaactacttccatctgccctacctggagcgaaagccctgcatctacatcaagagctggtggccggaccagcgccgccgcctctacaatgccaacatcatggaccacattgccgacaagctggtaagtatcaaggttacaagacaggtttaaggagaccaatagaaactgggcttgtcgagacagagaagactcttgcgtttctgggattttgccgatttcggcctattggttaaaaaatgagctgatttaacaaaaatttaacgcgaattttaacaaaatcacgtgcggaccgagcggccgcaggaacccctagtgatggagttggccactccctctctgcgcgctcgctcgctcactgaggccgggcgaccaaaggtcgcccgacgcccgggctttgcccgggcggcctcagtgagcgagcgagcgcgcagctgcctgcaggggcgcctgatgcggtattttctccttacgcatctgtgcggtatttcacaccgcatacgtcaaagcaaccatagtacgcgccctgtagcggcgcattaagcgcggcgggtgtggtggttacgcgcagcgtgaccgctacacttgccagcgccctagcgcccgctcctttcgctttcttcccttcctttctcgccacgttcgccggctttccccgtcaagctctaaatcgggggctccctttagggttccgatttagtgctttacggcacctcgaccccaaaaaacttgatttgggtgatggttcacgtagtgggccatcgccctgatagacggtttttcgccctttgacgttggagtccacgttctttaatagtggactcttgttccaaactggaacaacactcaaccctatctcgggctattcttttgatttataagggattttgccgatttcggcctattggttaaaaaatgagctgatttaacaaaaatttaacgcgaattttaacaaaatattaacgtttacaattttatggtgcactctcagtacaatctgctctgatgccgcatagttaagccagccccgacacccgccaacacccgctgacgcgccctgacgggcttgtctgctcccggcatccgcttacagacaagctgtgaccgtctccgggagctgcatgtgtcagaggttttcaccgtcatcaccgaaacgcgcgagacgaaagggcctcgtgatacgcctatttttataggttaatgtcatgataataatggtttcttagacgtcaggtggcacttttcggggaaatgtgcgcggaacccctatttgtttatttttctaaatacattcaaatatgtatccgctcatgagacaataaccctgataaatgcttcaa